European Patent Application EP 4 446 411 A1, published October 16, 2024. Title: VARIANT SUBTILISIN PROTEASES. Applicant: PEACCEL. Application EP. The sequence listing filed with the application follows.

SEQUENCE LISTING (9 sequences)

SEQ ID NO: 1 - protein, 4 aa, synthetic construct
AAPF

SEQ ID NO: 2 - protein, 269 aa, Bacillus subtilis
  source 1..269: note = wild-type subtilisin
AQSVPWGISRVQAPAAHNRGLTGSGVKVAVLDTGISTHPDLNIRGGASFVPGEPSTQDGNGHGTHVAGTIAALNNSIGVLGVAPSAELYAVKVLGASGSGSVSSIAQGLEWAGNNGMHVANLSLGSPSPSATLEQAVNSATSRGVLVVAASGNSGAGSISYPARYANAMAVGATDQNNNRASFSQYGAGLDIVAPGVNVQSTYPGSTYASLNGTSMATPHVAGAAALVKQKNPSWSNVQIRNHLKNTATSLGSTNLYGSGLVNAEAATR

SEQ ID NO: 3 - protein, 269 aa, synthetic construct
  source 1..269: note = variant subtilisin of WO1995010591
AQSVPWGISRVQAPAAHNRGLTGSGVKVAVLDTGISTHPDLNIRGGASFVPGEPSTQDGNGHGTHVAGTIAALDNSIGVLGVAPSAELYAVKVLGASGSGAWSSIAQGLEWAGNNGMHVANLSLGSPSPSATLEQAVNSATSRGVLVVAASGNSGAGSISYPARYANAMAVGATDQNNNRASFSQYGAGLDIVAPGVNVQSTYPGSTYASLNGTSMATPHVAGAAALVKQKNPSWSNVQIRNHLKNTATSLGSTNLYGSGLVNAEAATR

SEQ ID NO: 4 - protein, 269 aa, synthetic construct
  source 1..269: note = variant subtilisin
AQSVPWGISRVQAPAAHNRGLTGSGVKVAVLDTGISTHPDLNIRGGASFVPGEPSTQDGNGHGTHVAGTIAALDNSIGVLGVAPSAELYAVKVLGASGGGSWSSIAQGLEWAGNNGMHVANLSLGGPSPSATLEQAVNSATSRGVLVVAASGNSGAGSISYPARYANAMAVGATDQNNNRASFSQYGAGLEIVAPGVGVQSTYPGSTYASLSGTSMATPHVAGAAALVKQKNPSWSNVQIRNHLKNTATSLGSPNLYGSGLVNAEAATR

SEQ ID NO: 5 - protein, 269 aa, synthetic construct
  source 1..269: note = subtilisin variant
AQSVPWGISRVQAPAAHNRGLTGSGVKVAVLDTGISTHPDLNIRGGASFVPGEPSTQDGNGHGTHVAGTIAALDNSIGVLGVAPSAELYAVKVLGASGGGSWSSIAQGLEWAGNNGMHVANLSLGGPSPSATLEQAVNSATSRGVLVVAASGNSGAGSISYPARYANAMAVGATDQNNNRASFSQYGAGLDIVAPGVAVQSTYPGSTYASLSGTSMATPHVAGAAALVKQKNPSWSNVQIRNHLKNTATSLGSPNLYGSGLVNAEAATR

SEQ ID NO: 6 - protein, 269 aa, synthetic construct
  source 1..269: note = variant subtilisin
AQSVPWGISRVQAPAAHNRGLTGSGVKVAVLDTGISTHPDLNIRGGASFVPGEPSTQDGNGHGTHVAGTIAALDNSIGVLGVAPSAELYAVKVLGADGSGSVSSIAQGLEWAGNNGMHVANLSLGGPSPSATLEQAVNSATSRGVLVVAASGNSGAGSISYPARYANAMAVGATDQNNNRASFSQYGAGLDIVAPGVNVQSTYIGSTYASLNGTSMATPHVAGAAALVKQKNPSWSNVQIRNHLKNTATSLGSPNLYGNGLVNAEAATR

SEQ ID NO: 7 - DNA, 1140 bp, synthetic construct
  source 1..1140: mol_type = other DNA
  mat_peptide 334..1140
atgaagaaaccgttggggaaaattgtcgcaagcaccgcactactcatttctgttgcttttagttcatcgatcgcatcggctgctgaagaagcaaaagaaaaatatttaattggctttaatgagcaggaagctgtcagtgagtttgtagaacaagtagaggcaaatgacgaggtcgccattctctctgaggaagaggaagtcgaaattgaattgcttcatgaatttgaaacgattcctgttttatccgttgagttaagcccagaagatgtggacgcgcttgaactcgatccagcgatttcttatattgaagaggatgcagaagtaacgacaatggcgcaatcagtgccatggggaattagccgtgtgcaagccccagctgcccataaccgtggattgacaggttctggtgtaaaagttgctgtcctcgatacaggtatttccactcatccagacttaaatattcgtggtggcgctagctttgtaccaggggaaccatccactcaagatgggaatgggcatggcacgcatgtggccgggacgattgctgctttagacaattcgattggcgttcttggcgtagcgccgagcgcggaactatacgctgttaaagtattaggggcgagcggtggaggttcgtggagctcgattgcccaaggattggaatgggcagggaacaatggcatgcacgttgctaatttgagtttaggaggaccttcgccaagtgccacacttgagcaagctgttaatagcgcgacttctagaggcgttcttgttgtagcggcatctgggaattcaggtgcaggctcaatcagctatccggcccgttatgcgaacgcaatggcagtcggagctactgaccaaaacaacaaccgcgccagcttttcacagtatggcgcagggcttgaaattgtcgcaccaggtgtaggagtgcagagcacatacccaggttcaacgtatgccagcttatcaggtacatcgatggctactcctcatgttgcaggtgcagcagcccttgttaaacaaaagaacccatcttggtccaatgtacaaatccgcaatcatctaaagaatacggcaacgagcttaggaagccctaacttgtatggaagcggacttgtcaatgcagaagcggcaacacgc

SEQ ID NO: 8 - DNA, 1140 bp, synthetic construct
  source 1..1140: mol_type = other DNA
  mat_peptide 334..1140
atgaagaaaccgttggggaaaattgtcgcaagcaccgcactactcatttctgttgcttttagttcatcgatcgcatcggctgctgaagaagcaaaagaaaaatatttaattggctttaatgagcaggaagctgtcagtgagtttgtagaacaagtagaggcaaatgacgaggtcgccattctctctgaggaagaggaagtcgaaattgaattgcttcatgaatttgaaacgattcctgttttatccgttgagttaagcccagaagatgtggacgcgcttgaactcgatccagcgatttcttatattgaagaggatgcagaagtaacgacaatggcgcaatcagtgccatggggaattagccgtgtgcaagccccagctgcccataaccgtggattgacaggttctggtgtaaaagttgctgtcctcgatacaggtatttccactcatccagacttaaatattcgtggtggcgctagctttgtaccaggggaaccatccactcaagatgggaatgggcatggcacgcatgtggccgggacgattgctgctttagacaattcgattggcgttcttggcgtagcgccgagcgcggaactatacgctgttaaagtattaggggcgagcggtggaggttcgtggagctcgattgcccaaggattggaatgggcagggaacaatggcatgcacgttgctaatttgagtttaggaggaccttcgccaagtgccacacttgagcaagctgttaatagcgcgacttctagaggcgttcttgttgtagcggcatctgggaattcaggtgcaggctcaatcagctatccggcccgttatgcgaacgcaatggcagtcggagctactgaccaaaacaacaaccgcgccagcttttcacagtatggcgcagggcttgacattgtcgcaccaggtgtagccgtgcagagcacatacccaggttcaacgtatgccagcttatcaggtacatcgatggctactcctcatgttgcaggtgcagcagcccttgttaaacaaaagaacccatcttggtccaatgtacaaatccgcaatcatctaaagaatacggcaacgagcttaggaagccctaacttgtatggaagcggacttgtcaatgcagaagcggcaacacgc

SEQ ID NO: 9 - DNA, 1140 bp, synthetic construct
  source 1..1140: mol_type = other DNA
  mat_peptide 334..1140
atgaagaaaccgttggggaaaattgtcgcaagcaccgcactactcatttctgttgcttttagttcatcgatcgcatcggctgctgaagaagcaaaagaaaaatatttaattggctttaatgagcaggaagctgtcagtgagtttgtagaacaagtagaggcaaatgacgaggtcgccattctctctgaggaagaggaagtcgaaattgaattgcttcatgaatttgaaacgattcctgttttatccgttgagttaagcccagaagatgtggacgcgcttgaactcgatccagcgatttcttatattgaagaggatgcagaagtaacgacaatggcgcaatcagtgccatggggaattagccgtgtgcaagccccagctgcccataaccgtggattgacaggttctggtgtaaaagttgctgtcctcgatacaggtatttccactcatccagacttaaatattcgtggtggcgctagctttgtaccaggggaaccatccactcaagatgggaatgggcatggcacgcatgtggccgggacgattgctgctttagacaattcgattggcgttcttggcgtagcgccgagcgcggaactatacgctgttaaagtattaggggcggacggttcaggttcggtcagctcgattgcccaaggattggaatgggcagggaacaatggcatgcacgttgctaatttgagtttaggaggaccttcgccaagtgccacacttgagcaagctgttaatagcgcgacttctagaggcgttcttgttgtagcggcatctgggaattcaggtgcaggctcaatcagctatccggcccgttatgcgaacgcaatggcagtcggagctactgaccaaaacaacaaccgcgccagcttttcacagtatggcgcagggcttgacattgtcgcaccaggtgtaaacgtgcagagcacatacatcggttcaacgtatgccagcttaaacggtacatcgatggctactcctcatgttgcaggtgcagcagcccttgttaaacaaaagaacccatcttggtccaatgtacaaatccgcaatcatctaaagaatacggcaacgagcttaggaagccctaacttgtatggaaatggacttgtcaatgcagaagcggcaacacgc